European Patent Application EP 4 803 627 A1, published September 9, 2026. Title: Aptamers for nuclear translocation. Applicant: FUNDACION PARA LA INVESTIGACION MEDICA APLICADA. Application EP. The sequence listing filed with the application follows.

SEQUENCE LISTING (176 sequences)

SEQ ID NO: 1 - DNA, 45 bp, Synthetic construct
  source 1..45: mol_type = other DNA
ccgcctgtgtcttacctaatgttgcgtcatctctgtgcgtcacga

SEQ ID NO: 2 - DNA, 45 bp, Synthetic construct
  source 1..45: mol_type = other DNA
gcacaccacatcatactgtgtccaaccgttttgcgagtcctcccg

SEQ ID NO: 3 - DNA, 45 bp, Synthetic construct
  source 1..45: mol_type = other DNA
tggtgtgtgtgcttatccctttctttggtcggttgctgcgttttg

SEQ ID NO: 4 - DNA, 45 bp, Synthetic construct
  source 1..45: mol_type = other DNA
caaaccacgacataccttttccgttccaggcaggtctttattccg

SEQ ID NO: 5 - DNA, 45 bp, Synthetic construct
  source 1..45: mol_type = other DNA
ccccaccgctcaccatagtcactctcattgtccaacctctcactc

SEQ ID NO: 6 - DNA, 45 bp, Synthetic construct
  source 1..45: mol_type = other DNA
ccacacatccaaccgtaaatgctccttgtccagcaacccttaccg

SEQ ID NO: 7 - DNA, 45 bp, Synthetic construct
  source 1..45: mol_type = other DNA
caacacacatttcctcccccggcactgctggtcgattcgcgcggt

SEQ ID NO: 8 - DNA, 45 bp, Synthetic construct
  source 1..45: mol_type = other DNA
ggttatgtgggtggtgctgctgtgatggtgatgcgtccgatgggg

SEQ ID NO: 9 - DNA, 45 bp, Synthetic construct
  source 1..45: mol_type = other DNA
cacaactgaacacattgctgcacgtcttgatccctagctggttgc

SEQ ID NO: 10 - DNA, 45 bp, Synthetic construct
  source 1..45: mol_type = other DNA
acaacgcctctcttcttcttgccctgagaacacacacactacccg

SEQ ID NO: 11 - DNA, 45 bp, Synthetic construct
  source 1..45: mol_type = other DNA
acacacaccatgcttctttgccctttctctcttttgcttcccctg

SEQ ID NO: 12 - DNA, 45 bp, Synthetic construct
  source 1..45: mol_type = other DNA
acaacaattacccgtagtccagcatccgacgttctcctgccctcg

SEQ ID NO: 13 - DNA, 45 bp, Synthetic construct
  source 1..45: mol_type = other DNA
ccaccaacactcgtcatgctttggtcatctctgccccatgctgcg

SEQ ID NO: 14 - DNA, 45 bp, Synthetic construct
  source 1..45: mol_type = other DNA
aacccaccactcactctgcttgtttgcccgatgctgccctacctg

SEQ ID NO: 15 - DNA, 45 bp, Synthetic construct
  source 1..45: mol_type = other DNA
accaactcgcgtcctcacaacctgtctgcgtcctttcccatgctg

SEQ ID NO: 16 - DNA, 45 bp, Synthetic construct
  source 1..45: mol_type = other DNA
cagtgcgttatcccatgctgcgtttcaacatgatgcgtcttcgtg

SEQ ID NO: 17 - DNA, 45 bp, Synthetic construct
  source 1..45: mol_type = other DNA
acaccacacaccacacaccactcctgatctttgggactcgcctgt

SEQ ID NO: 18 - DNA, 45 bp, Synthetic construct
  source 1..45: mol_type = other DNA
cacaggcgatcatcactgctgctgtctatcattatgctgcgttcg

SEQ ID NO: 19 - DNA, 45 bp, Synthetic construct
  source 1..45: mol_type = other DNA
caacatcatcacgtgtccagtctatgctgctgcttcccccttccg

SEQ ID NO: 20 - DNA, 45 bp, Synthetic construct
  source 1..45: mol_type = other DNA
accccctgctgtcatttgtgcaagtcacttattcgctgcgcacga

SEQ ID NO: 21 - DNA, 45 bp, Synthetic construct
  source 1..45: mol_type = other DNA
ccggtccaaatccccaacgtgttttgttgctgccttttgtccccg

SEQ ID NO: 22 - DNA, 45 bp, Synthetic construct
  source 1..45: mol_type = other DNA
acaccaaactgcacatcttgcttgtgtccagcccctatgtatccg

SEQ ID NO: 23 - DNA, 45 bp, Synthetic construct
  source 1..45: mol_type = other DNA
cccatacgtgtccaacctttcccacaatgtgctgtcgttataccg

SEQ ID NO: 24 - DNA, 45 bp, Synthetic construct
  source 1..45: mol_type = other DNA
ccgtgtctgtctgttatacgtgtccatacaaaacactctggatcg

SEQ ID NO: 25 - DNA, 45 bp, Synthetic construct
  source 1..45: mol_type = other DNA
cacacacaatgagcgtcaatcgtatctttcaaatcttgctgcgtc

SEQ ID NO: 26 - DNA, 45 bp, Synthetic construct
  source 1..45: mol_type = other DNA
cgcacacaatctacctgtccataccgcacaccttctgttactccg

SEQ ID NO: 27 - DNA, 45 bp, Synthetic construct
  source 1..45: mol_type = other DNA
ccacgcattgtccaccgcagcacaattcactatttaccttccccg

SEQ ID NO: 28 - DNA, 45 bp, Synthetic construct
  source 1..45: mol_type = other DNA
tcactaatactgaccgtggacacattacactctggaggatcactc

SEQ ID NO: 29 - DNA, 45 bp, Synthetic construct
  source 1..45: mol_type = other DNA
acacatcatgcttaccctttacctgtccacaacctcccgttactc

SEQ ID NO: 30 - DNA, 45 bp, Synthetic construct
  source 1..45: mol_type = other DNA
ccaccccacatgatcgtccctctgatcgtcactccttactgctgt

SEQ ID NO: 31 - DNA, 45 bp, Synthetic construct
  source 1..45: mol_type = other DNA
gatgtcgacgcaccgttccacaccattcttttcctccatgcactc

SEQ ID NO: 32 - DNA, 45 bp, Synthetic construct
  source 1..45: mol_type = other DNA
tcaacccacattacactgtgtctacccgcccacattccttccctc

SEQ ID NO: 33 - DNA, 45 bp, Synthetic construct
  source 1..45: mol_type = other DNA
ccacacccatatgctgttttgtccaggcgatcaaacgtctcacgg

SEQ ID NO: 34 - DNA, 45 bp, Synthetic construct
  source 1..45: mol_type = other DNA
ggccgtcgcgaaaccatgatgtctgtcactctcatcgcgttactc

SEQ ID NO: 35 - DNA, 45 bp, Synthetic construct
  source 1..45: mol_type = other DNA
acacacactttctcactgcctcttttccctgctctcgcattcggt

SEQ ID NO: 36 - DNA, 45 bp, Synthetic construct
  source 1..45: mol_type = other DNA
gcataatcctcaccgtccacgaacaaattctttcgcactctggta

SEQ ID NO: 37 - DNA, 45 bp, Synthetic construct
  source 1..45: mol_type = other DNA
gccaatccgttcgcactgtgaccagacgccctttactcatatccg

SEQ ID NO: 38 - DNA, 45 bp, Synthetic construct
  source 1..45: mol_type = other DNA
gcagatcgtaccattttcgtccaaccgcgcataacctccttaccg

SEQ ID NO: 39 - DNA, 45 bp, Synthetic construct
  source 1..45: mol_type = other DNA
cccgacaacatgctgcttcttttgtactgtgcgtcactagatggt

SEQ ID NO: 40 - DNA, 45 bp, Synthetic construct
  source 1..45: mol_type = other DNA
acaatggctgtatcccacctgtccacacattcttgtcactctgcc

SEQ ID NO: 41 - DNA, 45 bp, Synthetic construct
  source 1..45: mol_type = other DNA
cgatcccacgcatattacatgtcactctgtttccgtcgctctggt

SEQ ID NO: 42 - DNA, 45 bp, Synthetic construct
  source 1..45: mol_type = other DNA
tggggggttgcttgcgttctggtatgttgttgctgcgttgagtgc

SEQ ID NO: 43 - DNA, 45 bp, Synthetic construct
  source 1..45: mol_type = other DNA
cgatcgtaggtgtggtgatgctgcctttttatgctgcgtccgacg

SEQ ID NO: 44 - DNA, 45 bp, Synthetic construct
  source 1..45: mol_type = other DNA
atacccggtccgatgctgcttacttctttgtcggtgatgcgtcta

SEQ ID NO: 45 - DNA, 45 bp, Synthetic construct
  source 1..45: mol_type = other DNA
tgaccctctctcgtgtccagccttattccttgctgtcgacctccg

SEQ ID NO: 46 - DNA, 45 bp, Synthetic construct
  source 1..45: mol_type = other DNA
cacacacacacgcatctcaacttgctgtcatcttctcccttaccg

SEQ ID NO: 47 - DNA, 45 bp, Synthetic construct
  source 1..45: mol_type = other DNA
gcacatcctcacatacttttgtccagcaaccaacacttcattccg

SEQ ID NO: 48 - DNA, 45 bp, Synthetic construct
  source 1..45: mol_type = other DNA
gggatacgtggttgctgcttatggtgggtgctgcactttaacttg

SEQ ID NO: 49 - DNA, 45 bp, Synthetic construct
  source 1..45: mol_type = other DNA
tgccatcctgtccaccatgtctctgagaaggtgctgcgtattgta

SEQ ID NO: 50 - DNA, 45 bp, Synthetic construct
  source 1..45: mol_type = other DNA
aacaccccactgccacttgtcctttgtcggtgctgcgttttggcg

SEQ ID NO: 51 - DNA, 45 bp, Synthetic construct
  source 1..45: mol_type = other DNA
acatcataacagtgtccaaccccgatattcactcattgttacccg

SEQ ID NO: 52 - DNA, 45 bp, Synthetic construct
  source 1..45: mol_type = other DNA
accaactcgcgtcctcacaacctgtctgcgtcttttcccatgctg

SEQ ID NO: 53 - DNA, 44 bp, Synthetic construct
  source 1..44: mol_type = other DNA
cacgctccatgctcgttcactaccgaaatgcacgttactctgtg

SEQ ID NO: 54 - DNA, 45 bp, Synthetic construct
  source 1..45: mol_type = other DNA
ccaccgtcgacattctgataccgtcactctttcctactgctgcgg

SEQ ID NO: 55 - DNA, 44 bp, Synthetic construct
  source 1..44: mol_type = other DNA
ccccgaacatgctgccaccttattgttgctcccatgctgcacta

SEQ ID NO: 56 - DNA, 45 bp, Synthetic construct
  source 1..45: mol_type = other DNA
caacatcatcacgtgtccagtctatgctgctgctttccccttccg

SEQ ID NO: 57 - DNA, 44 bp, Synthetic construct
  source 1..44: mol_type = other DNA
gggatggtccaccacacacacactctttttgcctccatttgacg

SEQ ID NO: 58 - DNA, 45 bp, Synthetic construct
  source 1..45: mol_type = other DNA
cgtgtccagaccgattttatcccaaactgctgcccctactacgcg

SEQ ID NO: 59 - DNA, 45 bp, Synthetic construct
  source 1..45: mol_type = other DNA
acaaacacatcctcctctttgtccacaaaacactcattctcatcg

SEQ ID NO: 60 - DNA, 45 bp, Synthetic construct
  source 1..45: mol_type = other DNA
ccaaccatgccttgattgtcactctctcttgctgcgtctaccgac

SEQ ID NO: 61 - DNA, 45 bp, Synthetic construct
  source 1..45: mol_type = other DNA
tgaccttaacgtgtccacccacaaaatgtctcgtccttcctactc

SEQ ID NO: 62 - DNA, 45 bp, Synthetic construct
  source 1..45: mol_type = other DNA
cacattgcccttcgttaccgttccacccaacccctttatcacccg

SEQ ID NO: 63 - DNA, 45 bp, Synthetic construct
  source 1..45: mol_type = other DNA
acaccgaacgcttttgatcttgtgtccaagcgcgccttccttccg

SEQ ID NO: 64 - DNA, 45 bp, Synthetic construct
  source 1..45: mol_type = other DNA
ccaccctcactccatgctcgcgtctaaattgcatgttgttgcgcc

SEQ ID NO: 65 - DNA, 45 bp, Synthetic construct
  source 1..45: mol_type = other DNA
cctcgccccatgccttgtcacttcatcatcgtctattgctgcgtt

SEQ ID NO: 66 - DNA, 45 bp, Synthetic construct
  source 1..45: mol_type = other DNA
acaccgttccacaagtcctcctccaccgtttcaacctcttcactc

SEQ ID NO: 67 - DNA, 45 bp, Synthetic construct
  source 1..45: mol_type = other DNA
gccgcatccaccgttccacctcaccccgttttccttgatgccatc

SEQ ID NO: 68 - DNA, 45 bp, Synthetic construct
  source 1..45: mol_type = other DNA
acccaccccgtatcttcgtgtccaccacccttcactctttaccct

SEQ ID NO: 69 - DNA, 45 bp, Synthetic construct
  source 1..45: mol_type = other DNA
cacaggcgatcatcactgctgctgtctatcatcatgctgcgttcg

SEQ ID NO: 70 - DNA, 45 bp, Synthetic construct
  source 1..45: mol_type = other DNA
acacccgatactgtgtccaaccgcaatcctttgttaactcatccg

SEQ ID NO: 71 - DNA, 45 bp, Synthetic construct
  source 1..45: mol_type = other DNA
taggcacctgtccatccaacattcagtcactctatctcatgcacg

SEQ ID NO: 72 - DNA, 45 bp, Synthetic construct
  source 1..45: mol_type = other DNA
aacaccacctcaccactgtagtccatcaccatccgtctatctccg

SEQ ID NO: 73 - DNA, 45 bp, Synthetic construct
  source 1..45: mol_type = other DNA
cacacacacacttcggcatttgtctattctctctttttggtcggg

SEQ ID NO: 74 - DNA, 45 bp, Synthetic construct
  source 1..45: mol_type = other DNA
acccgaactactatcccgttggtccacaaccgcgaatattccccc

SEQ ID NO: 75 - DNA, 45 bp, Synthetic construct
  source 1..45: mol_type = other DNA
ccccgccatgcctttatctgtcatctctgatttctgctgctgcgt

SEQ ID NO: 76 - DNA, 45 bp, Synthetic construct
  source 1..45: mol_type = other DNA
ccacacaccacacatgctctcgtacttgaccttctcgcgaactgg

SEQ ID NO: 77 - DNA, 45 bp, Synthetic construct
  source 1..45: mol_type = other DNA
tggcccacaccttctgtctgtccacacacacattctcctcgtttc

SEQ ID NO: 78 - DNA, 45 bp, Synthetic construct
  source 1..45: mol_type = other DNA
caaccacatgctgttttacacaaacctcgcgccatttctctcacg

SEQ ID NO: 79 - DNA, 45 bp, Synthetic construct
  source 1..45: mol_type = other DNA
acgtggccaccaaagctcattgtgtccaaccctttatcctatccg

SEQ ID NO: 80 - DNA, 45 bp, Synthetic construct
  source 1..45: mol_type = other DNA
ccgtgccaaccctgttatttactcgtgttgttgctcgtcgtcccg

SEQ ID NO: 81 - DNA, 45 bp, Synthetic construct
  source 1..45: mol_type = other DNA
acaaacacaccatgctgcattttcgactgtgcgtctttctgtagt

SEQ ID NO: 82 - DNA, 45 bp, Synthetic construct
  source 1..45: mol_type = other DNA
ccagctgcactcgtcatgctcgtcacgtgtttgctgctcacgttg

SEQ ID NO: 83 - DNA, 45 bp, Synthetic construct
  source 1..45: mol_type = other DNA
cagcccatgcattgattagtgtccagacccagtaccgttccatcg

SEQ ID NO: 84 - DNA, 45 bp, Synthetic construct
  source 1..45: mol_type = other DNA
ccgcccactgctcgtcatagactctttgttgctgcgttgttaatg

SEQ ID NO: 85 - DNA, 45 bp, Synthetic construct
  source 1..45: mol_type = other DNA
gacaacatctcgtgtccaaagcccgattcgaccctttgttttccg

SEQ ID NO: 86 - DNA, 45 bp, Synthetic construct
  source 1..45: mol_type = other DNA
ccgaactccatgctgtcctcgtcattgttgctgctgactcttcgt

SEQ ID NO: 87 - DNA, 45 bp, Synthetic construct
  source 1..45: mol_type = other DNA
acaatggccgtatcccacctgtccacacattcttgtcactctgcc

SEQ ID NO: 88 - DNA, 45 bp, Synthetic construct
  source 1..45: mol_type = other DNA
tcaccacacacacgctttcatggcttctccctatgcatcctcgac

SEQ ID NO: 89 - DNA, 45 bp, Synthetic construct
  source 1..45: mol_type = other DNA
cctcacgcgtacccatgctgctatatccgtcatgctgcttatcgt

SEQ ID NO: 90 - DNA, 45 bp, Synthetic construct
  source 1..45: mol_type = other DNA
accgtgatgtctgttcgtgtccaaaccttttccattctgtctccg

SEQ ID NO: 91 - DNA, 45 bp, Synthetic construct
  source 1..45: mol_type = other DNA
ccgtggacagtcccaccttatcgtctgtctccgtcattctgcccg

SEQ ID NO: 92 - DNA, 45 bp, Synthetic construct
  source 1..45: mol_type = other DNA
tatgttcggggttaacgtgtccaaccaccattgtcatctcctccg

SEQ ID NO: 93 - DNA, 45 bp, Synthetic construct
  source 1..45: mol_type = other DNA
cacacacctgcccctcttgatcacatctcgttgctgcggtttggg

SEQ ID NO: 94 - DNA, 45 bp, Synthetic construct
  source 1..45: mol_type = other DNA
ccacaacccgactgctcgtccaatcttgctgtcactcttggttgg

SEQ ID NO: 95 - DNA, 45 bp, Synthetic construct
  source 1..45: mol_type = other DNA
tggggctgagtgcgtcatcttccatggcttagttgctgcgtttgg

SEQ ID NO: 96 - DNA, 45 bp, Synthetic construct
  source 1..45: mol_type = other DNA
cacaaccaacacaacatcgtcacctcgtattcccactctcgatgc

SEQ ID NO: 97 - DNA, 45 bp, Synthetic construct
  source 1..45: mol_type = other DNA
accgctcaaaacccatgctgctcgtatacaactgcctgctgctcc

SEQ ID NO: 98 - DNA, 45 bp, Synthetic construct
  source 1..45: mol_type = other DNA
tctcccaccccctgctgcttttgacaatgctgctctgatcgttga

SEQ ID NO: 99 - DNA, 45 bp, Synthetic construct
  source 1..45: mol_type = other DNA
tggcgaggattggtgatgcgtcctattatgcgtgctgcttcatcg

SEQ ID NO: 100 - DNA, 45 bp, Synthetic construct
  source 1..45: mol_type = other DNA
ccgccaccaccttactttgtcactcctgatatgtctgctgcggtt

SEQ ID NO: 101 - DNA, 45 bp, Synthetic construct
  source 1..45: mol_type = other DNA
cacaccaaacgcccgccttatactcactctgttgccctgctgctc

SEQ ID NO: 102 - DNA, 45 bp, Synthetic construct
  source 1..45: mol_type = other DNA
caacacaccactcagtgtccaaacgtctcatttatcgtcactccg

SEQ ID NO: 103 - DNA, 45 bp, Synthetic construct
  source 1..45: mol_type = other DNA
ccctctcagaccatttgctgttccctcagtcacgtcatgctgctc

SEQ ID NO: 104 - DNA, 45 bp, Synthetic construct
  source 1..45: mol_type = other DNA
ccacatactcctgtcccgtcaactcgcttctaaccctgctgcgcc

SEQ ID NO: 105 - DNA, 45 bp, Synthetic construct
  source 1..45: mol_type = other DNA
ccacacatgctgatcatcattttcgcgcactcctttcctgctgcc

SEQ ID NO: 106 - DNA, 45 bp, Synthetic construct
  source 1..45: mol_type = other DNA
tcgcccccctaagccacataccctgctcgtcactcactcgtcacg

SEQ ID NO: 107 - DNA, 45 bp, Synthetic construct
  source 1..45: mol_type = other DNA
ccccaacataatgtctctctggcacatgctgcgttagatgttgtg

SEQ ID NO: 108 - DNA, 45 bp, Synthetic construct
  source 1..45: mol_type = other DNA
cagaacaaatgataatcgtgtccagccaatcccacttcctttccg

SEQ ID NO: 109 - DNA, 45 bp, Synthetic construct
  source 1..45: mol_type = other DNA
gcgaaatccccccatgctgtattgcccgaccatctgcgtcttccg

SEQ ID NO: 110 - DNA, 45 bp, Synthetic construct
  source 1..45: mol_type = other DNA
tggggacaggtgctgcttaaattatttgggatgctgcgctgtagt

SEQ ID NO: 111 - DNA, 45 bp, Synthetic construct
  source 1..45: mol_type = other DNA
taatgtacgtgtccaacccaatgctttatggcccacacaaatccg

SEQ ID NO: 112 - DNA, 45 bp, Synthetic construct
  source 1..45: mol_type = other DNA
acccccatgctgttcccttatgtcctgctgtgttttttgtctacg

SEQ ID NO: 113 - DNA, 45 bp, Synthetic construct
  source 1..45: mol_type = other DNA
cgcgccatcacctttgcttcgttactctccgtcaatgctgcggtt

SEQ ID NO: 114 - DNA, 45 bp, Synthetic construct
  source 1..45: mol_type = other DNA
tccccacaccacgatcttcacttttcgctcactctgtcgtacggc

SEQ ID NO: 115 - DNA, 45 bp, Synthetic construct
  source 1..45: mol_type = other DNA
tgaccataaccgcattgtcaattgtccacaccctttcactctgac

SEQ ID NO: 116 - DNA, 45 bp, Synthetic construct
  source 1..45: mol_type = other DNA
caccgattccagcacaacttggcatttgcgtcatctccctcactc

SEQ ID NO: 117 - DNA, 45 bp, Synthetic construct
  source 1..45: mol_type = other DNA
ccccacccacatctgtcgtcgttgttgctgttgttttggtttgtg

SEQ ID NO: 118 - DNA, 45 bp, Synthetic construct
  source 1..45: mol_type = other DNA
taccaacaccctccacctgccaacacaaccctttatgtctcatcg

SEQ ID NO: 119 - DNA, 45 bp, Synthetic construct
  source 1..45: mol_type = other DNA
tgtcccacacatcatcaccttgtccaagcgcgtttgtccttaccg

SEQ ID NO: 120 - DNA, 45 bp, Synthetic construct
  source 1..45: mol_type = other DNA
tcggacccatcccaccgtgccatactacacacattttctcctccg

SEQ ID NO: 121 - DNA, 45 bp, Synthetic construct
  source 1..45: mol_type = other DNA
acacgcaacttctcatagtgtccacccaacttctcgctcactacc

SEQ ID NO: 122 - DNA, 45 bp, Synthetic construct
  source 1..45: mol_type = other DNA
ggaccaccgttgtaccaaacccagctttcatcggcactctgatcg

SEQ ID NO: 123 - DNA, 45 bp, Synthetic construct
  source 1..45: mol_type = other DNA
ccacgctttaccaccaatcacactgctgctcctggttttcgatgc

SEQ ID NO: 124 - DNA, 45 bp, Synthetic construct
  source 1..45: mol_type = other DNA
cgacgccataatgctgctgttcttgatacctgctgcggttgggac

SEQ ID NO: 125 - DNA, 45 bp, Synthetic construct
  source 1..45: mol_type = other DNA
caacatcaagcatctcaccatctgtccagacgttttgccttcccg

SEQ ID NO: 126 - DNA, 45 bp, Synthetic construct
  source 1..45: mol_type = other DNA
acacccacccaatgctttaactttgccttttccacaattcgcggt

SEQ ID NO: 127 - DNA, 45 bp, Synthetic construct
  source 1..45: mol_type = other DNA
gggatcagtccgtgtccaccaattttcctattgtcacttccactc

SEQ ID NO: 128 - DNA, 45 bp, Synthetic construct
  source 1..45: mol_type = other DNA
ggcccagtactttccaccgtccatccgaccctattctatttaccg

SEQ ID NO: 129 - DNA, 45 bp, Synthetic construct
  source 1..45: mol_type = other DNA
cgatgcacaacctgccgatgcgtccttttgttgtttgctgcggtg

SEQ ID NO: 130 - DNA, 45 bp, Synthetic construct
  source 1..45: mol_type = other DNA
cacacatcaccatgctgttttgttaaggttgtcgtacatgcgggt

SEQ ID NO: 131 - DNA, 45 bp, Synthetic construct
  source 1..45: mol_type = other DNA
cacaccacgctatatgcacacacaactcaatcttattatcgcggt

SEQ ID NO: 132 - DNA, 45 bp, Synthetic construct
  source 1..45: mol_type = other DNA
accgaccaacatgctgctcatcaatcctgttctcctcgatcctgc

SEQ ID NO: 133 - DNA, 45 bp, Synthetic construct
  source 1..45: mol_type = other DNA
acaacaattacccgtagtccagcatccgacgttctcttgccctcg

SEQ ID NO: 134 - DNA, 45 bp, Synthetic construct
  source 1..45: mol_type = other DNA
ccaccgccatgctggtttcctcgttcgatgctgatcttgttgggg

SEQ ID NO: 135 - DNA, 45 bp, Synthetic construct
  source 1..45: mol_type = other DNA
gtggtgggtgtgctgtttcactggtttctatggtgtggtgcgtcc

SEQ ID NO: 136 - DNA, 45 bp, Synthetic construct
  source 1..45: mol_type = other DNA
cacacacacacgcccttccatttacgagtttgacttactccctcc

SEQ ID NO: 137 - DNA, 45 bp, Synthetic construct
  source 1..45: mol_type = other DNA
gggtgtgtgctgacttagttttgttgctgctctttttgtgcggtc

SEQ ID NO: 138 - DNA, 45 bp, Synthetic construct
  source 1..45: mol_type = other DNA
cactgccccatgctggtcttgttgaaacatgctgcgttttcatcg

SEQ ID NO: 139 - DNA, 45 bp, Synthetic construct
  source 1..45: mol_type = other DNA
gcacatcctcacatacctttgtccagcaaccaacacttcattccg

SEQ ID NO: 140 - DNA, 45 bp, Synthetic construct
  source 1..45: mol_type = other DNA
cccacattaccgaacccactgtccaaaagcatgtttcgttctccg

SEQ ID NO: 141 - DNA, 45 bp, Synthetic construct
  source 1..45: mol_type = other DNA
cacaccaccattgctgtttttgacctggaacgacttgcatgcggc

SEQ ID NO: 142 - DNA, 45 bp, Synthetic construct
  source 1..45: mol_type = other DNA
taccatacttcacctgtccaccaacccacaccctatacgccctcg

SEQ ID NO: 143 - DNA, 45 bp, Synthetic construct
  source 1..45: mol_type = other DNA
gccaaccacgccatacatgctgtcttttgatttgtgatgcgtccg

SEQ ID NO: 144 - DNA, 45 bp, Synthetic construct
  source 1..45: mol_type = other DNA
ttaccacccgatgagtaccgtgtctaatcccgcatcattcctccg

SEQ ID NO: 145 - DNA, 45 bp, Synthetic construct
  source 1..45: mol_type = other DNA
acaggactcacgtgtccaaccatttgttctccctatgttcccacg

SEQ ID NO: 146 - DNA, 45 bp, Synthetic construct
  source 1..45: mol_type = other DNA
ccacacgcacacaaactcatgacgaattgcacttgtttttccggt

SEQ ID NO: 147 - DNA, 45 bp, Synthetic construct
  source 1..45: mol_type = other DNA
tcaacatcatgcactattgtccaaacgcgctacttgcttcccacc

SEQ ID NO: 148 - DNA, 45 bp, Synthetic construct
  source 1..45: mol_type = other DNA
ccacaaccccgacatttcactctattcatcgatcctgctgcgagg

SEQ ID NO: 149 - DNA, 45 bp, Synthetic construct
  source 1..45: mol_type = other DNA
acaacaattacccgtagtccagcatccgacgttttcctgccctcg

SEQ ID NO: 150 - DNA, 45 bp, Synthetic construct
  source 1..45: mol_type = other DNA
cgtgtccagaccgattttattccaaactgctgcccctactacgcg

SEQ ID NO: 151 - DNA, 45 bp, Synthetic construct
  source 1..45: mol_type = other DNA
caacacccacaaccttcttgtcaaccttttcatcgcgcgaatttg

SEQ ID NO: 152 - skipped

SEQ ID NO: 153 - DNA, 133 bp, Synthetic construct
  source 1..133: mol_type = other DNA
agggccaggctccccagcaggcagaagtatgcaaagcatgcatctcaattagtcagcaaccaatccactcaggattggttgctgactaattgagatgcatgctttgcatacttctgcctgctggggagcctgg

SEQ ID NO: 154 - DNA, 143 bp, Synthetic construct
  source 1..143: mol_type = other DNA
agggccaggctccccagcaggcagaagtatgcaaagcatgcatctcaattagtcagcaaccacatccattaactcataatggatgtggttgctgactaattgagatgcatgctttgcatacttctgcctgctggggagcctgg

SEQ ID NO: 155 - DNA, 109 bp, Synthetic construct
  source 1..109: mol_type = other DNA
agggctggggactttccagcctggggactttccagctgggactttccaggatccactcaggatcctggaaagtcccagctggaaagtccccaggctggaaagtccccag

SEQ ID NO: 156 - skipped

SEQ ID NO: 157 - DNA, 18 bp, Synthetic construct
  source 1..18: mol_type = other DNA
atccagagtgacgcagca

SEQ ID NO: 158 - DNA, 18 bp, Synthetic construct
  source 1..18: mol_type = other DNA
tggacacggtggcttagt

SEQ ID NO: 159 - DNA, 105 bp, Synthetic construct
  source 1..105: mol_type = other DNA
agggagagagaaaatccagagtgacgcagcaccgcctgtgtcttacctaatgttgcgtcatctctgtgcgtcacgatggacacggtggcttagtaaaatctctct

SEQ ID NO: 160 - DNA, 105 bp, Synthetic construct
  source 1..105: mol_type = other DNA
agggagagagaaaatccagagtgacgcagcagcacaccacatcatactgtgtccaaccgttttgcgagtcctcccgtggacacggtggcttagtaaaatctctct

SEQ ID NO: 161 - DNA, 105 bp, Synthetic construct
  source 1..105: mol_type = other DNA
agggagagagaaaatccagagtgacgcagcatggtgtgtgtgcttatccctttctttggtcggttgctgcgttttgtggacacggtggcttagtaaaatctctct

SEQ ID NO: 162 - DNA, 105 bp, Synthetic construct
  source 1..105: mol_type = other DNA
agggagagagaaaatccagagtgacgcagcacaaaccacgacataccttttccgttccaggcaggtctttattccgtggacacggtggcttagtaaaatctctct

SEQ ID NO: 163 - DNA, 105 bp, Synthetic construct
  source 1..105: mol_type = other DNA
agggagagagaaaatccagagtgacgcagcaccccaccgctcaccatagtcactctcattgtccaacctctcactctggacacggtggcttagtaaaatctctct

SEQ ID NO: 164 - DNA, 105 bp, Synthetic construct
  source 1..105: mol_type = other DNA
agggagagagaaaatccagagtgacgcagcaccacacatccaaccgtaaatgctccttgtccagcaacccttaccgtggacacggtggcttagtaaaatctctct

SEQ ID NO: 165 - DNA, 105 bp, Synthetic construct
  source 1..105: mol_type = other DNA
agggagagagaaaatccagagtgacgcagcacaacacacatttcctcccccggcactgctggtcgattcgcgcggttggacacggtggcttagtaaaatctctct

SEQ ID NO: 166 - DNA, 105 bp, Synthetic construct
  source 1..105: mol_type = other DNA
agggagagagaaaatccagagtgacgcagcaggttatgtgggtggtgctgctgtgatggtgatgcgtccgatggggtggacacggtggcttagtaaaatctctct

SEQ ID NO: 167 - DNA, 105 bp, Synthetic construct
  source 1..105: mol_type = other DNA
agggagagagaaaatccagagtgacgcagcacacaactgaacacattgctgcacgtcttgatccctagctggttgctggacacggtggcttagtaaaatctctct

SEQ ID NO: 168 - DNA, 105 bp, Synthetic construct
  source 1..105: mol_type = other DNA
agggagagagaaaatccagagtgacgcagcaacaacgcctctcttcttcttgccctgagaacacacacactacccgtggacacggtggcttagtaaaatctctct

SEQ ID NO: 169 - DNA, 105 bp, Synthetic construct
  source 1..105: mol_type = other DNA
agggagagagaaaatccagagtgacgcagcaacacacaccatgcttctttgccctttctctcttttgcttcccctgtggacacggtggcttagtaaaatctctct

SEQ ID NO: 170 - DNA, 105 bp, Synthetic construct
  source 1..105: mol_type = other DNA
agggagagagaaaatccagagtgacgcagcaacaacaattacccgtagtccagcatccgacgttctcctgccctcgtggacacggtggcttagtaaaatctctct

SEQ ID NO: 171 - DNA, 16 bp, Synthetic construct
  source 1..16: mol_type = other DNA
tactggttgcaggatt

SEQ ID NO: 172 - DNA, 16 bp, Synthetic construct
  source 1..16: mol_type = other DNA
taagcactttggaaag

SEQ ID NO: 173 - DNA, 1801 bp, Synthetic construct
  source 1..1801: mol_type = other DNA
ggtctcgccctgatttaaatcgtcgaccgttacataacttacggtaaatggcccgcctggctgaccgcccaacgacccccgcccattgacgtcaataatgacgtatgttcccatagtaacgccaatagggactttccattgacgtcaatgggtggagtatttacggtaaactgcccacttggcagtacatcaagtgtatcatatgccaagtacgccccctattgacgtcaatgacggtaaatggcccgcctggcattatgcccagtacatgaccttatgggactttcctacttggcagtacatctacgtattagtcatcgctattaccatggtgatgcggttttggcagtacatcaatgggcgtggatagcggtttgactcacggggatttccaagtctccaccccattgacgtcaatgggagtttgttttggcaccaaaatcaacgggactttccaaaatgtcgtaacaactccgccccattgacgcaaatgggcggtaggcgtgtacggtgggaggtctatataagcagagctcgtttagtgaaccgtcagatcgcctggagacgccatccacgctgttttgacctccatagaagacaccgggaccgatccagcctccggactctagaggatccggtactcgaggaactgaaaaaccagaaagttaactggtaagtttagtctttttgtcttttatttcaggtcccggatccggtggtggtgcaaatcaaagaactgctcctcagtggatgttgcctttacttctaggcctgtacggaagtgttacttctgctctaaaagctgcggaattgtacccgcggcccgggatccaccggtcgccaccatggtgagcaagggcgaggagctgttcaccggggtggtgcccatcctggtcgagctggacggcgacgtaaacggccacaagttcagcgtgtccggcgagggcgagggcgatgccacctacggcaagctgaccctgaagttcatctgcaccaccggcaagctgcccgtgccctggcccaccctcgtgaccaccctgacctacggcgtgcagtgcttcagccgctaccccgaccacatgaagcagcacgacttcttcaagtccgccatgcccgaaggctacgtccaggagcgcaccatcttcttcaaggacgacggcaactacaagacccgcgccgaggtgaagttcgagggcgacaccctggtgaaccgcatcgagctgaagggcatcgacttcaaggaggacggcaacatcctggggcacaagctggagtacaactacaacagccacaacgtctatatcatggccgacaagcagaagaacggcatcaaggtgaacttcaagatccgccacaacatcgaggacggcagcgtgcagctcgccgaccactaccagcagaacacccccatcggcgacggccccgtgctgctgcccgacaaccactacctgagcacccagtccgccctgagcaaagaccccaacgagaagcgcgatcacatggtcctgctggagttcgtgaccgccgccgggatcactctcggcatggacgagctgtacaagtaaagcggccgcggggatccagacatgataagatacattgatgagtttggacaaaccacaactagaatgcagtgaaaaaaatgctttatttgtgaaatttgtgatgctattgctttatttgtaaccattataagctgcaataaacaagttaacaacaacaattgcattcattttatgtttcaggttcagggggaggtgtgggaggttttttagtcgaccatttaaatcggtctcgaggg

SEQ ID NO: 174 - DNA, 1857 bp, Synthetic construct
  source 1..1857: mol_type = other DNA
gcgtataatggactattgtgtgctgataggtctcgccctgatttaaatcgtcgaccgttacataacttacggtaaatggcccgcctggctgaccgcccaacgacccccgcccattgacgtcaataatgacgtatgttcccatagtaacgccaatagggactttccattgacgtcaatgggtggagtatttacggtaaactgcccacttggcagtacatcaagtgtatcatatgccaagtacgccccctattgacgtcaatgacggtaaatggcccgcctggcattatgcccagtacatgaccttatgggactttcctacttggcagtacatctacgtattagtcatcgctattaccatggtgatgcggttttggcagtacatcaatgggcgtggatagcggtttgactcacggggatttccaagtctccaccccattgacgtcaatgggagtttgttttggcaccaaaatcaacgggactttccaaaatgtcgtaacaactccgccccattgacgcaaatgggcggtaggcgtgtacggtgggaggtctatataagcagagctcgtttagtgaaccgtcagatcgcctggagacgccatccacgctgttttgacctccatagaagacaccgggaccgatccagcctccggactctagaggatccggtactcgaggaactgaaaaaccagaaagttaactggtaagtttagtctttttgtcttttatttcaggtcccggatccggtggtggtgcaaatcaaagaactgctcctcagtggatgttgcctttacttctaggcctgtacggaagtgttacttctgctctaaaagctgcggaattgtacccgcggcccgggatccaccggtcgccaccatggtgagcaagggcgaggagctgttcaccggggtggtgcccatcctggtcgagctggacggcgacgtaaacggccacaagttcagcgtgtccggcgagggcgagggcgatgccacctacggcaagctgaccctgaagttcatctgcaccaccggcaagctgcccgtgccctggcccaccctcgtgaccaccctgacctacggcgtgcagtgcttcagccgctaccccgaccacatgaagcagcacgacttcttcaagtccgccatgcccgaaggctacgtccaggagcgcaccatcttcttcaaggacgacggcaactacaagacccgcgccgaggtgaagttcgagggcgacaccctggtgaaccgcatcgagctgaagggcatcgacttcaaggaggacggcaacatcctggggcacaagctggagtacaactacaacagccacaacgtctatatcatggccgacaagcagaagaacggcatcaaggtgaacttcaagatccgccacaacatcgaggacggcagcgtgcagctcgccgaccactaccagcagaacacccccatcggcgacggccccgtgctgctgcccgacaaccactacctgagcacccagtccgccctgagcaaagaccccaacgagaagcgcgatcacatggtcctgctggagttcgtgaccgccgccgggatcactctcggcatggacgagctgtacaagtaaagcggccgcggggatccagacatgataagatacattgatgagtttggacaaaccacaactagaatgcagtgaaaaaaatgctttatttgtgaaatttgtgatgctattgctttatttgtaaccattataagctgcaataaacaagttaacaacaacaattgcattcattttatgtttcaggttcagggggaggtgtgggaggttttttagtcgaccatttaaatcggtctcgagggtatcagcacacaattgcccattatacgc

SEQ ID NO: 175 - DNA, 18 bp, Synthetic construct
  source 1..18: mol_type = other DNA
atccagagtgacgcagca

SEQ ID NO: 176 - DNA, 18 bp, Synthetic construct
  source 1..18: mol_type = other DNA
actaagccaccgtgtcca